European Patent Application EP 4 122 484 A1, published January 25, 2023. Title: COMPOSITION HAVING ANTIHYPERTENSIVE EFFECT COMPRISING CHP (CYCLO-HIS PRO). Applicant: NOVMETAPHARMA CO., LTD. SEOUL NATIONAL UNIVERSITY HOSPITALSEOUL NATIONAL UNIVERSITY HOSPITAL SNU R&DB FOUNDATION. The sequence listing filed with the application follows.

SEQUENCE LISTING (4 sequences)

SEQ ID NO: 1 - DNA, 20 bp, Artificial
  eNOS forward primer
cccggaaagagggattgtgt

SEQ ID NO: 2 - DNA, 20 bp, Artificial
  eNOS reverse primer
tgcaaccaatgctgtaggca

SEQ ID NO: 3 - DNA, 18 bp, Artificial
  β-actin forward primer
gggaaggtgacagcattg

SEQ ID NO: 4 - DNA, 23 bp, Artificial
  β-actin reverse primer
atgaagtattaaggcggaagatt